European Patent Specification EP 4 392 555 B1, published August 5, 2026. Title: METHODS AND COMPOSITIONS FOR DETECTING GENOMIC METHYLATION. Applicant: Illumina, Inc. The sequence listing filed with the application follows.

SEQUENCE LISTING (26 sequences)

SEQ ID NO: 1 - DNA, 14 bp, synthetic construct
  misc_feature 1..14: note = A14
  source 1..14: mol_type = other DNA
tcgtcggcagcgtc

SEQ ID NO: 2 - DNA, 14 bp, synthetic construct
  misc_feature 1..14: note = A14 prime
  source 1..14: mol_type = other DNA
gacgctgccgacga

SEQ ID NO: 3 - DNA, 14 bp, synthetic construct
  misc_feature 1..14: note = Converted-A14
  source 1..14: mol_type = other DNA
ttgttggtagtgtt

SEQ ID NO: 4 - DNA, 14 bp, synthetic construct
  misc_feature 1..14: note = (Converted-A14)prime
  source 1..14: mol_type = other DNA
aacactaccaacaa

SEQ ID NO: 5 - DNA, 14 bp, synthetic construct
  misc_feature 1..14: note = Converted-A14prime
  source 1..14: mol_type = other DNA
gatgttgttgatga

SEQ ID NO: 6 - DNA, 14 bp, synthetic construct
  misc_feature 1..14: note = (Converted-A14prime)prime
  source 1..14: mol_type = other DNA
tcatcaacaacatc

SEQ ID NO: 7 - DNA, 19 bp, synthetic construct
  misc_feature 1..19: note = ME
  source 1..19: mol_type = other DNA
agatgtgtataagagacag

SEQ ID NO: 8 - DNA, 19 bp, synthetic construct
  misc_feature 1..19: note = MEprime
  source 1..19: mol_type = other DNA
ctgtctcttatacacatct

SEQ ID NO: 9 - DNA, 19 bp, synthetic construct
  misc_feature 1..19: note = Converted- ME
  source 1..19: mol_type = other DNA
agatgtgtataagagatag

SEQ ID NO: 10 - DNA, 19 bp, synthetic construct
  misc_feature 1..19: note = (Converted- ME)prime
  source 1..19: mol_type = other DNA
ctatctcttatacacatct

SEQ ID NO: 11 - DNA, 19 bp, synthetic construct
  misc_feature 1..19: note = Converted- MEprime
  source 1..19: mol_type = other DNA
ttgttttttatatatattt

SEQ ID NO: 12 - DNA, 19 bp, synthetic construct
  misc_feature 1..19: note = (Converted- MEprime)prime
  source 1..19: mol_type = other DNA
aaatatatataaaaaacaa

SEQ ID NO: 13-18 - skipped (6 entries)

SEQ ID NO: 19 - DNA, 33 bp, synthetic construct
  misc_feature 1..33: note = Nextera Read1 primer (A14-ME)Tm = 64.5degreeC
  source 1..33: mol_type = other DNA
tcgtcggcagcgtcagatgtgtataagagacag

SEQ ID NO: 20 - DNA, 34 bp, synthetic construct
  misc_feature 1..34: note = Nextera Read2 primer (B14-ME)Tm = 64.2degreeC
  source 1..34: mol_type = other DNA
gtctcgtgggctcggagatgtgtataagagacag

SEQ ID NO: 21 - DNA, 41 bp, synthetic construct
  misc_feature 1..41: note = Custom Read2 primer (B8+convertedA14+ME)Tm = 64.8degreeC
  source 1..41: mol_type = other DNA
gggctcggttgttggtagtgttagatgtgtataagagacag

SEQ ID NO: 22 - DNA, 29 bp, synthetic construct
  misc_feature 1..29: note = P5
  source 1..29: mol_type = other DNA
aatgatacggcgaccaccgagatctacac

SEQ ID NO: 23 - DNA, 24 bp, synthetic construct
  misc_feature 1..24: note = P7
  source 1..24: mol_type = other DNA
caagcagaagacggcatacgagat

SEQ ID NO: 24 - DNA, 53 bp, synthetic construct
  misc_feature 1..53: note = Tailed index primer 1 (P7-X7index-B8-converted-A14)
  misc_feature 25..31: note = n = A,T,C or G
  source 1..53: mol_type = other DNA
caagcagaagacggcatacgagatnnnnnnngggctcggttgttggtagtgtt

SEQ ID NO: 25 - DNA, 48 bp, synthetic construct
  misc_feature 1..48: note = Tailed index primer 2 (P5-X5 index-A14)
  misc_feature 30..34: note = n = A,T,C or G
  source 1..48: mol_type = other DNA
aatgatacggcgaccaccgagatctacacnnnnntcgtcggcagcgtc

SEQ ID NO: 26 - DNA, 61 bp, synthetic construct
  misc_feature 1..61: note = First adapter comprising a hairpin, neck andcleavable site
  misc_feature 20: note = N = uracil (U)
  source 1..61: mol_type = other DNA
ctgtctcttatacacatctngggctcggtcgtcggcagcgtcagatgtgtataagagacag